European Patent Specification EP 3 098 233 B1, published November 6, 2024. Title: RETICULOCYTE GROWTH FACTOR AND PREPARING METHOD AND APPLICATION THEREOF. The sequence listing filed with the application follows.

SEQUENCE LISTING (1 sequence)

SEQ ID NO: 1 - protein, 418 aa, Homo sapiens
MPSSVSWGILLLAGLCCLVPVSLAEDPQGDAAQKTDTSHHDQDHPTFNKITPNLAEFAFSLYRQLAHQSNSTNIFFSPVSIATAFAMLSLGTKADTHDEILEGLNFNLTEIPEAQIHEGFQELLRTLNQPDSQLQLTTGNGLFLSEGLKLVDKFLEDVKKLYHSEAFTVNFGDTEEAKKQINDYVEKGTQGKIVDLVKELDRDTVFALVNYIFFKGKWERPFEVKDTEEEDFHVDQVTTVKVPMMKRLGMFNIQHCKKLSSWVLLMKYLGNATAIFFLPDEGKLQHLENELTHDIITKFLENEDRRSASLHLPKLSITGTYDLKSVLGQLGITKVFSNGADLSGVTEEAPLKLSKAVHKAVLTIDEKGTEAAGAMFLEAIPMSIPPEVKFNKPFVFLMIEQDTKSPLFMGKVVNPTQK